European Patent Specification EP 3 884 055 B1, published August 9, 2023. Title: DOUBLE AND INDUCIBLE SUICIDE GENE CONSTRUCT AND ITS USE IN GENE THERAPY. Applicant: Consejo Superior de Investigaciones Científicas (CSIC). The sequence listing filed with the application follows.

SEQUENCE LISTING (12 sequences)

SEQ ID NO: 1 - DNA, 1200 bp, Artificial Sequence
  Encoding nucleotide sequence for the icaspase9 protein
atgctcgagggagtgcaggtggaaaccatctccccaggagacgggcgcaccttccccaagcgcggccagacctgcgtggtgcactacaccgggatgcttgaagatggaaagaaagttgattcctcccgggacagaaacaagccctttaagtttatgctaggcaagcaggaggtgatccgaggctgggaagaaggggttgcccagatgagtgtgggtcagagagccaaactgactatatctccagattatgcctatggtgccactgggcacccaggcatcatcccaccacatgccactctcgtcttcgatgtggagcttctaaaactggaatctggcggtggatccggagtcgacggatttggtgatgtcggtgctcttgagagtttgaggggaaatgcagatttggcttacatcctgagcatggagccctgtggccactgcctcattatcaacaatgtgaacttctgccgtgagtccgggctccgcacccgcactggctccaacatcgactgtgagaagttgcggcgtcgcttctcctcgctgcatttcatggtggaggtgaagggcgacctgactgccaagaaaatggtgctggctttgctggagctggcgcagcaggaccacggtgctctggactgctgcgtggtggtcattctctctcacggctgtcaggccagccacctgcagttcccaggggctgtctacggcacagatggatgccctgtgtcggtcgagaagattgtgaacatcttcaatgggaccagctgccccagcctgggagggaagcccaagctctttttcatccaggcctgtggtggggagcagaaagaccatgggtttgaggtggcctccacttcccctgaagacgagtcccctggcagtaaccccgagccagatgccaccccgttccaggaaggtttgaggaccttcgaccagctggacgccatatctagtttgcccacacccagtgacatctttgtgtcctactctactttcccaggttttgtttcctggagggaccccaagagtggctcctggtacgttgagaccctggacgacatctttgagcagtgggctcactctgaagacctgcagtccctcctgcttagggtcgctaatgctgtttcggtgaaagggatttataaacagatgcctggttgctttaatttcctccggaaaaaacttttctttaaaacatca

SEQ ID NO: 2 - DNA, 1128 bp, Herpes simplex
atggcttcgtacccctgccatcaacacgcgtctgcgttcgaccaggctgcgcgttctcgcggccataacaaccgacgtacggcgttgcgccctcgccggcaacaaaaagccacggaagtccgcctggagcagaaaatgcccacgctactgcgggtttatatagacggtccccacgggatggggaaaaccaccaccacgcaactgctggtggccctgggttcgcgcgacgatatcgtctacgtacccgagccgatgacttactggcgggtgttgggggcttccgagacaatcgcgaacatctacaccacacaacaccgcctcgaccagggtgagatatcggccggggacgcggcggtggtaatgacaagcgcccagataacaatgggcatgccttatgccgtgaccgacgccgttctggctcctcatatcgggggggaggctgggagctcacatgccccgcccccggccctcaccctcatcttcgaccgccatcccatcgccgccctcctgtgctacccggccgcgcgataccttatgggcagcatgaccccccaggccgtgctggcgttcgtggccctcatcccgccgaccttgcccggcacaaacatcgtgttgggggcccttccggaggacagacacatcgaccgcctggccaaacgccagcgccccggcgagcggcttgacctggctatgctggccgcgattcgccgcgtttatgggctgcttgccaatacggtgcggtatctgcagggcggcgggtcgtggcgggaggattggggacagctttcgggggcggccgtgccgccccagggtgccgagccccagagcaacgcgggcccacgaccccatatcggggacacgttatttaccctgtttcgggcccccgagttgctggcccccaacggcgacctgtataacgtgtttgcctgggctttggacgtcttggccaaacgcctccgtcccatgcatgtctttatcctggattacgaccaatcgcccgccggctgccgggacgccctgctgcaacttacctccgggatggtccagacccacgtcaccaccccaggctccataccgacgatctgcgacctggcgcgcacgtttgcccgggagatgggggaggctaac

SEQ ID NO: 3 - DNA, 133 bp, Artificial Sequence
  Beta-globin intron
gtaagtatcaaggttacaagacaggtttaaggagaccaatagaaactgggcttgtcgagacagagaagactcttgcgtttctgataggcacctattggtcttactgacatccactttgcctttctctccacag

SEQ ID NO: 4 - protein, 400 aa, Artificial Sequence
  Amino acid sequence of icaspase9
MLEGVQVETISPGDGRTFPKRGQTCVVHYTGMLEDGKKVDSSRDRNKPFKFMLGKQEVIRGWEEGVAQMSVGQRAKLTISPDYAYGATGHPGIIPPHATLVFDVELLKLESGGGSGVDGFGDVGALESLRGNADLAYILSMEPCGHCLIINNVNFCRESGLRTRTGSNIDCEKLRRRFSSLHFMVEVKGDLTAKKMVLALLELAQQDHGALDCCVVVILSHGCQASHLQFPGAVYGTDGCPVSVEKIVNIFNGTSCPSLGGKPKLFFIQACGGEQKDHGFEVASTSPEDESPGSNPEPDATPFQEGLRTFDQLDAISSLPTPSDIFVSYSTFPGFVSWRDPKSGSWYVETLDDIFEQWAHSEDLQSLLLRVANAVSVKGIYKQMPGCFNFLRKKLFFKTS

SEQ ID NO: 5 - protein, 376 aa, Herpes simplex
MASYPCHQHASAFDQAARSRGHNNRRTALRPRRQQKATEVRLEQKMPTLLRVYIDGPHGMGKTTTTQLLVALGSRDDIVYVPEPMTYWRVLGASETIANIYTTQHRLDQGEISAGDAAVVMTSAQITMGMPYAVTDAVLAPHIGGEAGSSHAPPPALTLIFDRHPIAALLCYPAARYLMGSMTPQAVLAFVALIPPTLPGTNIVLGALPEDRHIDRLAKRQRPGERLDLAMLAAIRRVYGLLANTVRYLQGGGSWREDWGQLSGAAVPPQGAEPQSNAGPRPHIGDTLFTLFRAPELLAPNGDLYNVFAWALDVLAKRLRPMHVFILDYDQSPAGCRDALLQLTSGMVQTHVTTPGSIPTICDLARTFAREMGEAN

SEQ ID NO: 6 - DNA, 1388 bp, Artificial Sequence
  EF1alpha Promoter
gacattgattattgagtacatttatattggctcatgtccaacattaccgccatgagtaattcatacaaaaggactcgcccctgccttggggaatcccagggaccgtcgttaaactcccactaacgtagaacccagagatcgctgcgttcccgccccctcacccgcccgctctcgtcatcactgaggtggagaagagcatgcgtgaggctccggtgcccgtcagtgggcagagcgcacatcgcccacagtccccgagaagttggggggaggggtcggcaattgaaccggtgcctagagaaggtggcgcggggtaaactgggaaagtgatgtcgtgtactggctccgcctttttcccgagggtgggggagaaccgtatataagtgcagtagtcgccgtgaacgttctttttcgcaacgggtttgccgccagaacacaggtaagtgccgtgtgtggttcccgcgggcctggcctctttacgggttatggcccttgcgtgccttgaattacttccacgcccctggctgcagtacgtgattcttgatcccgagcttcgggttggaagtgggtgggagagttcgaggccttgcgcttaaggagccccttcgcctcgtgcttgagttgaggcctggcttgggcgctggggccgccgcgtgcgaatctggtggcaccttcgcgcctgtctcgctgctttcgataagtctctagccatttaaaatttttgatgacctgctgcgacgctttttttctggcaagatagtcttgtaaatgcgggccaagatctgcacactggtatttcggtttttggggccgcgggcggcgacggggcccgtgcgtcccagcgcacatgttcggcgaggcggggcctgcgagcgcggccaccgagaatcggacgggggtagtctcaagctggccggcctgctctggtgcctggcctcgcgccgccgtgtatcgccccgccctgggcggcaaggctggcccggtcggcaccagttgcgtgagcggaaagatggccgcttcccggccctgctgcagggagctcaaaatggaggacgcggcgctcgggagagcgggcgggtgagtcacccacacaaaggaaaagggcctttccgtcctcagccgtcgcttcatgtgactccacggagtaccgggcgccgtccaggcacctcgattagttctcgagcttttggagtacgtcgtctttaggttggggggaggggttttatgcgatggagtttccccacactgagtgggtggagactgaagttaggccagcttggcacttgatgtaattctccttggaatttgccctttttgagtttggatcttggttcattctcaagcctcagacagtggttcaaagtttttttcttccatttcaggtgtcgtga

SEQ ID NO: 7 - protein, 22 aa, Artificial Sequence
  T2A Element
ASRAEGRGSLLTCGDVEENPGP

SEQ ID NO: 8 - DNA, 66 bp, Artificial Sequence
  Encoding nucleotide sequence for the T2A element
gctagcagagccgagggcaggggaagtcttctaacatgcggggacgtggaggaaaatcccgggccc

SEQ ID NO: 9 - protein, 22 aa, Artificial Sequence
  P2A Element
GSGATNFSLLKQAGDVEENPGP

SEQ ID NO: 10 - DNA, 66 bp, Artificial Sequence
  Encoding nucleotide sequence for the P2A element
ggaagcggagctactaacttcagcctgctgaagcaggctggagacgtggaggagaaccctggacct

SEQ ID NO: 11 - DNA, 840 bp, Artificial Sequence
  Encoding gene for the truncated membrane receptor dNGFR
atgggggcaggtgccaccggccgcgccatggacgggccgcgcctgctgctgttgctgcttctgggggtgtcccttggaggtgccaaggaggcatgccccacaggcctgtacacacacagcggtgagtgctgcaaagcctgcaacctgggcgagggtgtggcccagccttgtggagccaaccagaccgtgtgtgagccctgcctggacagcgtgacgttctccgacgtggtgagcgcgaccgagccgtgcaagccgtgcaccgagtgcgtggggctccagagcatgtcggcgccgtgcgtggaggccgacgacgccgtgtgccgctgcgcctacggctactaccaggatgagacgactgggcgctgcgaggcgtgccgcgtgtgcgaggcgggctcgggcctcgtgttctcctgccaggacaagcagaacaccgtgtgcgaggagtgccccgacggcacgtattccgacgaggccaaccacgtggacccgtgcctgccctgcaccgtgtgcgaggacaccgagcgccagctccgcgagtgcacacgctgggccgacgccgagtgcgaggagatccctggccgttggattacacggtccacacccccagagggctcggacagcacagcccccagcacccaggagcctgaggcacctccagaacaagacctcatagccagcacggtggcaggtgtggtgaccacagtgatgggcagctcccagcccgtggtgacccgaggcaccaccgacaacctcatccctgtctattgctccatcctggctgctgtggttgtgggccttgtggcctacatagccttcaagaggtggaacagggggattctc

SEQ ID NO: 12 - protein, 280 aa, Artificial Sequence
  dNGFR truncated membrane receptor
MGAGATGRAMDGPRLLLLLLLGVSLGGAKEACPTGLYTHSGECCKACNLGEGVAQPCGANQTVCEPCLDSVTFSDVVSATEPCKPCTECVGLQSMSAPCVEADDAVCRCAYGYYQDETTGRCEACRVCEAGSGLVFSCQDKQNTVCEECPDGTYSDEANHVDPCLPCTVCEDTERQLRECTRWADAECEEIPGRWITRSTPPEGSDSTAPSTQEPEAPPEQDLIASTVAGVVTTVMGSSQPVVTRGTTDNLIPVYCSILAAVVVGLVAYIAFKRWNRGIL